European Patent Application EP 4 733 322 A1, published April 29, 2026. Title: 经修饰的TCR恒定区及其在TCR融合蛋白中的用途. Applicant: 北京可瑞生物科技有限公司. The sequence listing filed with the application follows.

SEQUENCE LISTING (101 sequences)

SEQ ID NO: 1 - protein, 91 aa, Homo sapiens
NIQNPDPAVYQLRDSKSSDKSVCLFTDFDSQTNVSQSKDSDVYITDKTVLDMRSMDFKSNSAVAWSNKSDFACANAFNNSIIPEDTFFPSP

SEQ ID NO: 2 - protein, 86 aa, synthetic construct
NIQKPDPAVYQLRDSKSSDKSVCLFTDFDSQTNVSQSKDSDVYITDKCVLDMRSMDFKSNSAVAWSNKSDFACANAFNNSIIPEDT

SEQ ID NO: 3 - protein, 86 aa, synthetic construct
NIQKPDPAVYRLRDSKSSDKSVCLFTDFDSQTNVSQSKDSDVYITDKCVLDMRSMDFKSNSAVAWSNKSDFACANAFNNSIIPEDT

SEQ ID NO: 4 - protein, 86 aa, Homo sapiens
NIQKPDPAVYQLRDSKSSDKIVCLFTDFDSQTNVSQSKDSDVYITDKCVLDMRSMDFKSNSAVAWSNKSDFACANAFNNSIIPEDT

SEQ ID NO: 5 - protein, 86 aa, synthetic construct
NIQKPDPAVYQLRDSKSSDKSVCLFTDFDSQTNVSQSKDSDVYITDPCVLDMRSMDFKSNSAVAWSNKSDFACANAFNNSIIPEDT

SEQ ID NO: 6 - protein, 86 aa, synthetic construct
NIQKPDPAVYQLRDSKSSDKSVCLFTDFDSQTNVSQSKDSDVYITDKCVLDMRDMDFKSNSAVAWSNKSDFACANAFNNSIIPEDT

SEQ ID NO: 7 - protein, 86 aa, synthetic construct
NIQKPDPAVYQLRDSKSSDKSVCLFTDFDSQTNVSQSKDSDVYITDKCVLDMREMDFKSNSAVAWSNKSDFACANAFNNSIIPEDT

SEQ ID NO: 8 - protein, 86 aa, synthetic construct
NIQKPDPAVYQLRDSKSSDKSVCLFTDFDSQTNVSQSKDSDVYITDKCVLDMRNMDFKSNSAVAWSNKSDFACANAFNNSIIPEDT

SEQ ID NO: 9 - protein, 86 aa, synthetic construct
NIQKPDPAVYQLRDSKSSDKSVCLFTDFDSQTNVSQSKDSDVYITDKCVLDMRSMDFKSNSAVAWSNKSDFACANAFNNSEIPEDT

SEQ ID NO: 10 - protein, 86 aa, synthetic construct
NIQKPDPAVYQLRDSKSSDKSVCLFTDFDSQTNVSQSKDSDVYITDPCVLDMRDMDFKSNSAVAWSNKSDFACANAFNNSIIPEDT

SEQ ID NO: 11 - protein, 86 aa, synthetic construct
NIQKPDPAVYQLRDSKSSDKIVCLFTDFDSQTNVSQSKDSDVYITDKCVLDMRDMDFKSNSAVAWSNKSDFACANAFNNSIIPEDT

SEQ ID NO: 12 - protein, 86 aa, synthetic construct
NIQKPDPAVYQLRDSKSSDKIVCLFTDFDSQTNVSQSKDSDVYITDPCVLDMRSMDFKSNSAVAWSNKSDFACANAFNNSIIPEDT

SEQ ID NO: 13 - protein, 86 aa, synthetic construct
NIQKPDPAVYQLRDSKSSDKIVCLFTDFDSQTNVSQSKDSDVYITDPCVLDMRDMDFKSNSAVAWSNKSDFACANAFNNSIIPEDT

SEQ ID NO: 14 - protein, 130 aa, synthetic construct
EDLKNVFPPEVAVFEPSEAEISHTQKATLVCLATGFYPDHVELSWWVNGKEVHSGVSTDPQPLKEQPALNDSRYCLSSRLRVSATFWQNPRNHFRCQVQFYGLSENDEWTQDRAKPVTQIVSAEAWGRAD

SEQ ID NO: 15 - protein, 130 aa, synthetic construct
EDLKNVFPPEVAVFEPSEAEISHTQKATLVCLATGFYPDHVELSWWVNGKEVHSGVCTDPQPLKEQPALNDSRYALSSRLRVSATFWQDPRNHFRCQVQFYGLSENDEWTQDRAKPVTQIVSAEAWGRAD

SEQ ID NO: 16 - protein, 130 aa, synthetic construct
EDLKNVFPPEVAVFEPSEAEISHTQKATLVCLATGFYPDHVELSWWVNGKEVHSGVCTDPQPLKEQPALNDSRYALSSRLRVPATFWQDPRNHFRCQVQFYGLSENDEWTQDRAKPVTQIVSAEAWGRAD

SEQ ID NO: 17 - protein, 130 aa, synthetic construct
EDLKNVFPPEVAVFEPSEAEISHTQKATLVCLATGFYPDHVELSWWVNGKEVHSGVCTDPQPLKEQPALNDSRYALSSRLRVEATFWQDPRNHFRCQVQFYGLSENDEWTQDRAKPVTQIVSAEAWGRAD

SEQ ID NO: 18 - protein, 130 aa, synthetic construct
EDLKNVFPPEVAVFEPSEAEISHTQKATLVCLATGFYPDHVELSWWVNGKEVHSGVCTDPQPLKEQPALNDSRYALSSRLRVDATFWQDPRNHFRCQVQFYGLSENDEWTQDRAKPVTQIVSAEAWGRAD

SEQ ID NO: 19 - protein, 130 aa, synthetic construct
EDLKNVFPPEVAVFEPSEAEISHTQKATLVCLATGFYPDHVELSWWVNGKEVHSGVCTDPQPLKEQPALNDSRYALSSRLRVLATFWQDPRNHFRCQVQFYGLSENDEWTQDRAKPVTQIVSAEAWGRAD

SEQ ID NO: 20 - protein, 130 aa, synthetic construct
EDLKNVFPPEVAVFEPSEAEISHTQKATLVCLATGFYPDHVELSWWVNGKEVHSGVCTDPQPLKEQPALNDSRYALSSRLRVNATFWQDPRNHFRCQVQFYGLSENDEWTQDRAKPVTQIVSAEAWGRAD

SEQ ID NO: 21 - protein, 130 aa, synthetic construct
EDLKNVFPPEVAVFEPSEAEISHTQKATLVCLATGFYPDHVELSWWVNGKEVHSGVCTDPQPLKEQPALNDSRYALSSRLRVSADFWQDPRNHFRCQVQFYGLSENDEWTQDRAKPVTQIVSAEAWGRAD

SEQ ID NO: 22 - protein, 130 aa, synthetic construct
EDLKNVFPPEVAVFEPSEAEISHTQKATLVCLATGFYPDHVELSWWVNGKEVHSGVCTDPQPLKEQPALNDSRYALSSRLRVSATFWQDPRNHFRCQVLFYGLSENDEWTQDRAKPVTQIVSAEAWGRAD

SEQ ID NO: 23 - protein, 130 aa, synthetic construct
EDLKNVFPPEVAVFEPSEAEISHTQKATLVCLATGFYPDHVELSWWVNGKEVHSGVCTDPQPLKEQPALNDSRYALSSRLRVSADFWQDPRNHFRCQVLFYGLSENDEWTQDRAKPVTQIVSAEAWGRAD

SEQ ID NO: 24 - protein, 112 aa, synthetic construct
RKEVEQDPGPFNVPEGATVAFNCTYSNSASQSFFWYRQDCRKEPKLLMSVYSSGNEDGRFTAQLNRASQYISLLIRDSKLSDSATYLCVVPGGTGGGNKLTFGTGTQLKVEL

SEQ ID NO: 25 - protein, 113 aa, synthetic construct
DTAVSQTPKYLVTQMGNDKSIKCEQNLGHDTMDWYKQDSKKFLKIMFSYNNKELIINETVPNRFSPKSPDKAHLNLHINSLELGDSAVYFCASSHWGAQETQYFGPGTRLLVL

SEQ ID NO: 26 - protein, 114 aa, synthetic construct
GESVGLHLPTLGVQEGDNSIINCAYSNSASDYFIWYKQESGKGPQFIIDIRSNMDKRQGQRVTVLLNKTVKHLSLQIAATQPGDSAVYFCAENSDGTSYGKLTFGQGTILTVHP

SEQ ID NO: 27 - protein, 115 aa, synthetic construct
EAGVAQSPRYKIIEKRQSVAFWCNPISGHATLYWYQQILGQGPKLLIQFQNNGVVDDSQLPKDRFSAERLKGVDSTLKIQPAKLEDSAVYLCASSLVGSPDYEQYFGPGTRLTVT

SEQ ID NO: 28 - protein, 117 aa, synthetic construct
AQSVAQPEDQVNVAEGNPLTVKCTYSVSGNPYLFWYVQYPNRGLQFLLKYITGDNLVKGSYGFEAEFNKSQTSFHLKKPSALVSDSALYFCAVRDIEGAGNNRKLIWGLGTSLAVNP

SEQ ID NO: 29 - protein, 113 aa, synthetic construct
DAGVIQSPRHEVTEMGQEVTLRCKPISGHNSLFWYRQTMMRGLELLIYFNNNVPIDDSGMPEDRFSAKMPNASFSTLKIQPSEPRDSAVYFCASSEGFYTEAFFGQGTRLTVV

SEQ ID NO: 30 - protein, 111 aa, synthetic construct
GEDVEQSLFLSVREGDSSVINCTYTDSSMTYLYWYKQEPGAGLQLLTYIFAFESMKQDQRLTVLLNKKDKHLSLRIADTQTGDSAIYFCAGSGGGTDKLIFGTGTRLQVFP

SEQ ID NO: 31 - protein, 117 aa, synthetic construct
GAVVSQHPSWVICKSGTSVKIECRSLDFEATTMFWYRQFPKQSLMLMATTDYGSKATYEQGVEKDKFLINHASLTLSTLTVTSAHPEDSSFYICSAREPGQGPWEQYFGPGTRLTVT

SEQ ID NO: 32 - protein, 111 aa, synthetic construct
GEDVEQSLFLSVREGDSSVINCTYTDSSMTYLYWYKQEPGAGLQLLTYIFFYQDMKQDQRLTVLLNKKDKHLSLRIADTQTGDSAIYFCAGSGGGTDKLIFGTGTRLQVFP

SEQ ID NO: 33 - protein, 117 aa, synthetic construct
GAVVSQHPSWVICKSGTSVKIECRSLDFEATTMFWYRQFPKQSLMLMATTDYGSKATYEQGVEKDKFLINHASLTLSTLTVTSAHPEDSSFYICSAREPGQAWSDQYFGPGTRLTVT

SEQ ID NO: 34 - protein, 107 aa, synthetic construct
RKEVEQDPGPFNVPEGATVAFNCTYSNSASQSFFWYRQDCRKEPKLLMSVYSSGNEDGRFTAQLNRASQYISLLIRDSKLSDSATYLCVVTNARLMFGDGTQLVVKP

SEQ ID NO: 35 - protein, 114 aa, synthetic construct
EAQVTQNPRYLITVTGKKLTVTCSQNMNHEYMSWYRQDPGLGLRQIYYSMNVEVTDKGDVPEGYKVSRKEKNFPLILESPSPNQTSLYFCASTSIVSSGRGEQFFGPGTRLTVL

SEQ ID NO: 36 - protein, 11 aa, synthetic construct
ANIGGGSGGGG

SEQ ID NO: 37 - protein, 9 aa, synthetic construct
GGGSGGGGD

SEQ ID NO: 38 - protein, 6 aa, synthetic construct
NSASQS

SEQ ID NO: 39 - protein, 6 aa, synthetic construct
VYSSGN

SEQ ID NO: 40 - protein, 13 aa, synthetic construct
VVPGGTGGGNKLT

SEQ ID NO: 41 - protein, 5 aa, synthetic construct
LGHDT

SEQ ID NO: 42 - protein, 6 aa, synthetic construct
YNNKEL

SEQ ID NO: 43 - protein, 12 aa, synthetic construct
ASSHWGAQETQY

SEQ ID NO: 44 - protein, 6 aa, synthetic construct
NSASDY

SEQ ID NO: 45 - protein, 7 aa, synthetic construct
IRSNMDK

SEQ ID NO: 46 - protein, 13 aa, synthetic construct
AENSDGTSYGKLT

SEQ ID NO: 47 - protein, 5 aa, synthetic construct
SGHAT

SEQ ID NO: 48 - protein, 6 aa, synthetic construct
FQNNGV

SEQ ID NO: 49 - protein, 13 aa, synthetic construct
ASSLVGSPDYEQY

SEQ ID NO: 50 - protein, 6 aa, synthetic construct
VSGNPY

SEQ ID NO: 51 - protein, 8 aa, synthetic construct
YITGDNLV

SEQ ID NO: 52 - protein, 15 aa, synthetic construct
AVRDIEGAGNNRKLI

SEQ ID NO: 53 - protein, 5 aa, synthetic construct
SGHNS

SEQ ID NO: 54 - protein, 6 aa, synthetic construct
FNNNVP

SEQ ID NO: 55 - protein, 11 aa, synthetic construct
ASSEGFYTEAF

SEQ ID NO: 56 - protein, 6 aa, synthetic construct
DSSMTY

SEQ ID NO: 57 - protein, 7 aa, synthetic construct
IFAFESM

SEQ ID NO: 58 - protein, 9 aa, synthetic construct
AGSGGGTDK

SEQ ID NO: 59 - protein, 6 aa, synthetic construct
DFEATT

SEQ ID NO: 60 - protein, 7 aa, synthetic construct
TDYGSKA

SEQ ID NO: 61 - protein, 11 aa, synthetic construct
SAREPGQGPWE

SEQ ID NO: 62 - protein, 6 aa, synthetic construct
DSSMTY

SEQ ID NO: 63 - protein, 7 aa, synthetic construct
IFFYQDM

SEQ ID NO: 64 - protein, 9 aa, synthetic construct
AGSGGGTDK

SEQ ID NO: 65 - protein, 6 aa, synthetic construct
DFEATT

SEQ ID NO: 66 - protein, 7 aa, synthetic construct
TDYGSKA

SEQ ID NO: 67 - protein, 11 aa, synthetic construct
SAREPGQAWSD

SEQ ID NO: 68 - protein, 112 aa, synthetic construct
GEDVEQSLFLSVREGDSSVINCTYTDSSSTYLYWYKQEPGAGLQLLTYIFSNMDMKQDQRLTVLLNKKDKHLSLRIADTQTGDSAIYFCAGSGGGTDKLIFGTGTRLQVFPN

SEQ ID NO: 69 - protein, 118 aa, synthetic construct
GAVVSQHPSWVICKSGTSVKIECRSLDFQATTMFWYRQFPKQSLMLMATSDYQTCVTYEQGVEKDKFLINHASLTLSTLTVTSAHPEDSSFYICSAREPGQGPFEQYFGPGTRLTVTE

SEQ ID NO: 70 - protein, 6 aa, synthetic construct
NSASQS

SEQ ID NO: 71 - protein, 6 aa, synthetic construct
VYSSGN

SEQ ID NO: 72 - protein, 10 aa, synthetic construct
AVISAGTALI

SEQ ID NO: 73 - protein, 5 aa, synthetic construct
SGHDT

SEQ ID NO: 74 - protein, 6 aa, synthetic construct
YYEEEE

SEQ ID NO: 75 - protein, 15 aa, synthetic construct
ASSLGWRGGLYTEAF

SEQ ID NO: 76 - protein, 109 aa, synthetic construct
RKEVEQDPGPFNVPEGATVAFNCTYSNSASQSFFWYRQDCRKEPKLLMSVYSSGNEDGRFTAQLNRASQYISLLIRDSKLSDSATYLCAVISAGTALIFGKGTTLSVSS

SEQ ID NO: 77 - protein, 116 aa, synthetic construct
DAGVTQSPTHLIKTRGQQVTLRCSPKSGHDTVSWYQQALGQGPQFIFQYYEEEERQRGNFPDRFSGHQFPNYSSELNVNALLLGDSALYLCASSLGWRGGLYTEAFFGQGTRLTVV

SEQ ID NO: 78 - protein, 6 aa, synthetic construct
NSASQS

SEQ ID NO: 79 - protein, 6 aa, synthetic construct
VYSSGN

SEQ ID NO: 80 - protein, 8 aa, synthetic construct
VVTNARLM

SEQ ID NO: 81 - protein, 5 aa, synthetic construct
MNHEY

SEQ ID NO: 82 - protein, 6 aa, synthetic construct
SMNVEV

SEQ ID NO: 83 - protein, 14 aa, synthetic construct
ASTSIVSSGRGEQF

SEQ ID NO: 84 - protein, 6 aa, synthetic construct
DRGSQS

SEQ ID NO: 85 - protein, 6 aa, synthetic construct
IYSNGD

SEQ ID NO: 86 - protein, 12 aa, synthetic construct
AVNLGAAGNKLT

SEQ ID NO: 87 - protein, 5 aa, synthetic construct
SGHAT

SEQ ID NO: 88 - protein, 6 aa, synthetic construct
FQNNGV

SEQ ID NO: 89 - protein, 13 aa, synthetic construct
ASSFSDSYNSPLH

SEQ ID NO: 90 - protein, 108 aa, synthetic construct
QKEVEQNSGPLSVPEGAIASLNCTYSDRGSQSFFWYRQYSGKSPELIMSIYSNGDKEDGRFTAQLNKASQYVSLLIRDSQPSDSATYLCAVNLGAAGNKLTFGGGTRV

SEQ ID NO: 91 - protein, 115 aa, synthetic construct
EAGVAQSPRYKIIEKRQSVAFWCNPISGHATLYWYQQILGQGPKLLIQFQNNGVVDDSQLPKDRFSAERLKGVDSTLKIQPAKLEDSAVYLCASSFSDSYNSPLHFGNGTRLTVT

SEQ ID NO: 92 - protein, 330 aa, synthetic construct
RKEVEQDPGPFNVPEGATVAFNCTYSNSASQSFFWYRQDCRKEPKLLMSVYSSGNEDGRFTAQLNRASQYISLLIRDSKLSDSATYLCVVPGGTGGGNKLTFGTGTQLKVELANIGGGSGGGGEVQLVESGGGLVQPGGSLRLSCAASGYSFTGYTMNWVRQAPGKCLEWVALINPYKGVSTYNQKFKDRFTISVDKSKNTAYLQMNSLRAEDTAVYYCARSGYYGDSDWYFDVWGQGTLVTVSSSQKPDPAVYQLRDSKSSDKIVCLFTDFDSQTNVSQSKDSDVYITDPCVLDMRDMDFKSNSAVAWSNKSDFACANAFNNSIIPEDT

SEQ ID NO: 93 - protein, 358 aa, synthetic construct
DIQMTQSPSSLSASVGDRVTITCRASQDIRNYLNWYQQKPGKAPKLLIYYTSRLESGVPSRFSGSGSGTDYTLTISSLQPEDFATYYCQQGNTLPWTFGCGTKVEIKGGGSGGGGDTAVSQTPKYLVTQMGNDKSIKCEQNLGHDTMDWYKQDSKKFLKIMFSYNNKELIINETVPNRFSPKSPDKAHLNLHINSLELGDSAVYFCASSHWGAQETQYFGPGTRLLVLEDLKNVFPPEVAVFEPSEAEISHTQKATLVCLATGFYPDHVELSWWVNGKEVHSGVCTDPQPLKEQPALNDSRYALSSRLRVSADFWQDPRNHFRCQVLFYGLSENDEWTQDRAKPVTQIVSAEAWGRAD

SEQ ID NO: 94 - protein, 108 aa, synthetic construct
SQQGEEDPQALSIQEGENATMNCSYKTSINNLQWYRQNSGRGLVHLILIRSNEREKHSGRLRVTLDTSKKSSSLLITASRAADTASYFCATDGSTPMQFGKGTRLSVI

SEQ ID NO: 95 - protein, 112 aa, synthetic construct
DGGITQSPKYLFRKEGQNVTLSCEQNLNHDAMYWYRQDPGQGLRLIYYSWAQGDFQKGDIAEGYSVSREKKESFPLTVTSAQKNPTAFYLCASSWGAPYEQYFGPGTRLTVT

SEQ ID NO: 96 - protein, 122 aa, synthetic construct
EVQLVESGGGLVQPGGSLRLSCAASGYSFTGYTMNWVRQAPGKCLEWVALINPYKGVSTYNQKFKDRFTISVDKSKNTAYLQMNSLRAEDTAVYYCARSGYYGDSDWYFDVWGQGTLVTVSS

SEQ ID NO: 97 - protein, 107 aa, synthetic construct
DIQMTQSPSSLSASVGDRVTITCRASQDIRNYLNWYQQKPGKAPKLLIYYTSRLESGVPSRFSGSGSGTDYTLTISSLQPEDFATYYCQQGNTLPWTFGCGTKVEIK

SEQ ID NO: 98 - protein, 10 aa, synthetic construct
GGGGSGGGGS

SEQ ID NO: 99 - protein, 15 aa, synthetic construct
GGGGSGGGGSGGGGS

SEQ ID NO: 100 - protein, 231 aa, synthetic construct
EPKSSDKTHTCPPCPAPPVAGPSVFLFPPKPKDTLMISRTPEVTCVVVDVSHEDPEVKFNWYVDGVEVHNAKTKPREEQYQSTYRVVSVLTVLHQDWLNGKEYKCKVSNKALPASIEKTISKAKGQPREPQVCTLPPSRDELTKNQVSLSCAVKGFYPSDIAVEWESNGQPENNYKTTPPVLDSDGSFFLVSKLTVDKSRWQQGNVFSCSVMHEALHNHYTQKSLSLSPGK

SEQ ID NO: 101 - protein, 231 aa, synthetic construct
EPKSSDKTHTCPPCPAPPVAGPSVFLFPPKPKDTLMISRTPEVTCVVVDVSHEDPEVKFNWYVDGVEVHNAKTKPREEQYQSTYRVVSVLTVLHQDWLNGKEYKCKVSNKALPASIEKTISKAKGQPREPQVYTLPPCRDELTKNQVSLWCLVKGFYPSDIAVEWESNGQPENNYKTTPPVLDSDGSFFLYSKLTVDKSRWQQGNVFSCSVMHEALHNHYTQKSLSLSPGK